European Patent Application EP 4 585 613 A1, published July 16, 2025. Title: METHOD FOR BIOSYNTHESIS OF HUMAN BODY STRUCTURAL MATERIAL TYPE-VIII COLLAGEN. Applicant: SHANXI JINBO BIO-PHARMACEUTICAL CO.,LTD. Application EP. The sequence listing filed with the application follows.

SEQUENCE LISTING (30 sequences)

SEQ ID NO: 1 - protein, 48 aa, Homo sapiens
GKPGMPGMPGKPGAMGMPGAKGEIGQKGEIGPMGIPGPQGPPGPHGLP

SEQ ID NO: 2 - protein, 288 aa, synthetic construct
GKPGMPGMPGKPGAMGMPGAKGEIGQKGEIGPMGIPGPQGPPGPHGLPGKPGMPGMPGKPGAMGMPGAKGEIGQKGEIGPMGIPGPQGPPGPHGLPGKPGMPGMPGKPGAMGMPGAKGEIGQKGEIGPMGIPGPQGPPGPHGLPGKPGMPGMPGKPGAMGMPGAKGEIGQKGEIGPMGIPGPQGPPGPHGLPGKPGMPGMPGKPGAMGMPGAKGEIGQKGEIGPMGIPGPQGPPGPHGLPGKPGMPGMPGKPGAMGMPGAKGEIGQKGEIGPMGIPGPQGPPGPHGLP

SEQ ID NO: 3 - DNA, 864 bp, synthetic construct
  source 1..864: mol_type = other DNA
gggaaacccggaatgccgggcatgccggggaagccgggtgcgatgggtatgccgggcgcgaaaggcgagatcggccagaagggcgaaattggcccgatgggtattccgggtccgcagggtccaccgggtccgcatggtctgccgggcaagccgggtatgccgggcatgccgggtaagccgggtgcaatgggtatgccgggcgcgaaaggtgaaatcggccaaaaaggtgagatcggcccgatgggtattccgggtccgcagggtcctccgggcccgcacggcctgcctggtaaaccgggtatgcccggcatgccgggcaagccgggtgcaatgggtatgccgggcgcgaaaggtgagatcggtcaaaaaggtgaaattggtccgatgggcattccgggtccgcagggcccaccgggtccgcacggcctgccgggtaagccgggtatgccggggatgccaggcaagccaggtgcgatgggtatgccgggcgcgaaaggtgaaattggtcagaaaggtgagatcggtccgatgggtattccgggtccgcaaggtccgcctggtccgcatggcttgccgggcaagccgggtatgccgggcatgccgggcaagccgggcgctatgggaatgcctggcgcgaaaggtgagatcggacaaaaaggcgaaatcggtccgatgggcatcccgggcccacagggtccaccgggtccccacggcctgccgggtaagccgggcatgccgggcatgccgggcaagccgggcgctatgggtatgccgggtgcgaaaggtgaaatcggccagaagggcgagatcggtccgatgggtattccgggcccacaaggtccgccgggcccacacggtttaccg

SEQ ID NO: 4 - protein, 42 aa, Homo sapiens
GKPGVTGFPGPQGPLGKPGAPGEPGPQGPIGVPGVQGPPGIP

SEQ ID NO: 5 - protein, 252 aa, synthetic construct
GKPGVTGFPGPQGPLGKPGAPGEPGPQGPIGVPGVQGPPGIPGKPGVTGFPGPQGPLGKPGAPGEPGPQGPIGVPGVQGPPGIPGKPGVTGFPGPQGPLGKPGAPGEPGPQGPIGVPGVQGPPGIPGKPGVTGFPGPQGPLGKPGAPGEPGPQGPIGVPGVQGPPGIPGKPGVTGFPGPQGPLGKPGAPGEPGPQGPIGVPGVQGPPGIPGKPGVTGFPGPQGPLGKPGAPGEPGPQGPIGVPGVQGPPGIP

SEQ ID NO: 6 - DNA, 756 bp, synthetic construct
  source 1..756: mol_type = other DNA
ggaaaacccggggtaactggttttccgggtccgcagggtccgctgggtaaaccgggtgcaccgggtgaaccgggcccgcaaggtcctattggtgtgccgggcgttcagggcccaccgggtattccgggcaagccgggcgtgacgggatttccgggtccgcaaggtccgttaggcaagccgggcgctccgggtgaaccgggtcctcaaggtccgatcggtgtgcctggcgtccagggtccaccgggtatcccgggcaaaccgggcgttaccggtttcccgggccctcaaggtccgctgggtaagccgggtgcgccgggcgagccaggcccacagggtccgattggtgtgccgggcgtgcaaggtccaccgggcattccgggcaaaccgggcgttaccggcttccccggtccgcagggtccgctgggcaagccgggcgcgccaggtgagccgggccctcaaggtccgatcggggtcccaggtgttcaaggcccgcctggcattccgggtaaaccgggcgttaccggctttccgggtccgcaaggtccgttgggtaaaccgggtgcccctggcgagccgggtccgcagggtcccatcggcgtgccgggtgttcagggtccgccgggcatcccgggtaaaccgggcgtgaccggtttcccgggtccgcagggtccgctgggtaagccgggtgcgccaggcgaaccgggcccgcagggtcccatcggtgttccgggtgtccagggcccaccgggcatcccg

SEQ ID NO: 7 - protein, 36 aa, Homo sapiens
GKPGGPGLPGQPGPKGDRGPKGLPGPQGLRGPKGDK

SEQ ID NO: 8 - protein, 216 aa, synthetic construct
GKPGGPGLPGQPGPKGDRGPKGLPGPQGLRGPKGDKGKPGGPGLPGQPGPKGDRGPKGLPGPQGLRGPKGDKGKPGGPGLPGQPGPKGDRGPKGLPGPQGLRGPKGDKGKPGGPGLPGQPGPKGDRGPKGLPGPQGLRGPKGDKGKPGGPGLPGQPGPKGDRGPKGLPGPQGLRGPKGDKGKPGGPGLPGQPGPKGDRGPKGLPGPQGLRGPKGDK

SEQ ID NO: 9 - DNA, 648 bp, synthetic construct
  source 1..648: mol_type = other DNA
gggaaacccggaggaccgggtctgccgggccaaccgggtccgaagggcgaccgcggtccgaagggtctgccgggcccacagggtctgcgtggtccaaaaggcgataaaggcaaaccgggtggtccgggccttccgggccagcctggcccaaagggcgatcgtggtccgaagggcttgccgggcccacagggtctgcgtggtccgaaaggtgacaagggcaaaccgggcggtccgggcctgccggggcaacctggccccaagggcgaccgcggtccgaagggtctgccgggtccgcaaggtctgcgcggtccgaagggtgataaaggcaaaccgggtggtccgggcctgccaggccagccgggtccgaagggcgatcgtggcccgaagggcttgccgggtccgcagggtttgagaggcccaaagggcgacaaaggtaaaccgggcggtccgggcctgccgggtcagccgggtccgaagggtgatcgtggtccgaaaggcctcccgggccctcaaggtctgcgtggtccgaagggcgacaaaggtaaaccgggcggtccgggtttgccgggtcaaccgggtccgaagggtgatcgcggtccgaaaggcctgccgggtccgcagggcttacgtggtccgaagggcgacaaa

SEQ ID NO: 10 - protein, 33 aa, Homo sapiens
GKPGQDGIPGQPGFPGGKGEQGLPGLPGPPGLP

SEQ ID NO: 11 - protein, 198 aa, synthetic construct
GKPGQDGIPGQPGFPGGKGEQGLPGLPGPPGLPGKPGQDGIPGQPGFPGGKGEQGLPGLPGPPGLPGKPGQDGIPGQPGFPGGKGEQGLPGLPGPPGLPGKPGQDGIPGQPGFPGGKGEQGLPGLPGPPGLPGKPGQDGIPGQPGFPGGKGEQGLPGLPGPPGLPGKPGQDGIPGQPGFPGGKGEQGLPGLPGPPGLP

SEQ ID NO: 12 - DNA, 594 bp, synthetic construct
  source 1..594: mol_type = other DNA
gggaaacccggacaagacggcattccgggtcaaccgggattcccgggtggcaaaggtgaacaaggtttgccaggcttgccaggtccgcctggcttgccgggcaaaccgggccaggatggcatcccgggccaaccgggctttccgggcggtaagggcgaacagggtttaccgggtctgccaggcccaccgggtctgccgggcaagccgggtcaagatggtattccgggtcagccgggttttccgggtggtaaaggtgagcagggtttgccggggctgccgggtccgccaggcctgccgggtaaaccgggtcaggatggtatcccgggtcaaccgggtttcccgggcggtaaaggcgagcagggtctgccgggccttccgggtcctccgggcctgccgggtaagccgggtcaggacggcatcccgggacaaccgggcttcccgggcggtaagggtgagcagggtctgccgggcctgccgggtccgcctggtctcccgggcaagccgggccaagacggcattccgggccagcctggctttccgggtggtaaaggtgaacagggcctgccgggcctgccgggtccgccaggcctgccg

SEQ ID NO: 13 - protein, 180 aa, Homo sapiens
GKPGFPGPKGDRGMGGVPGALGPRGEKGPIGAPGIGGPPGEPGLPGIPGPMGPPGAIGFPGPKGEGGIVGPQGPPGPKGEPGLQGFPGKPGFLGEVGPPGMRGLPGPIGPKGEAGQKGVPGLPGVPGLLGPKGEPGIPGDQGLQGPPGIPGIGGPSGPIGPPGIPGPKGEPGLPGPPGFP

SEQ ID NO: 14 - protein, 360 aa, synthetic construct
GKPGFPGPKGDRGMGGVPGALGPRGEKGPIGAPGIGGPPGEPGLPGIPGPMGPPGAIGFPGPKGEGGIVGPQGPPGPKGEPGLQGFPGKPGFLGEVGPPGMRGLPGPIGPKGEAGQKGVPGLPGVPGLLGPKGEPGIPGDQGLQGPPGIPGIGGPSGPIGPPGIPGPKGEPGLPGPPGFPGKPGFPGPKGDRGMGGVPGALGPRGEKGPIGAPGIGGPPGEPGLPGIPGPMGPPGAIGFPGPKGEGGIVGPQGPPGPKGEPGLQGFPGKPGFLGEVGPPGMRGLPGPIGPKGEAGQKGVPGLPGVPGLLGPKGEPGIPGDQGLQGPPGIPGIGGPSGPIGPPGIPGPKGEPGLPGPPGFP

SEQ ID NO: 15 - DNA, 1080 bp, synthetic construct
  source 1..1080: mol_type = other DNA
ggaaaacccgggttcccgggcccgaaaggtgaccgcggtatgggtggtgtcccgggcgcgctgggtccgcgtggtgagaaaggcccaatcggtgcccctggcattggcggcccgccaggcgaaccgggcctgccgggcattccgggtcctatgggcccgccgggcgcaattggtttcccgggccccaagggtgagggtggtatcgtgggcccacagggtccaccgggtccaaaaggtgagccgggccttcaaggtttcccggggaaaccgggttttctgggtgaagttggtccaccgggtatgcgcggtttgccgggtcccatcggtccgaagggcgaagcgggtcagaaaggtgtgccgggcttgccgggcgtgccgggcttgctgggtccgaagggcgaaccgggcattccgggtgatcagggtttacaaggtccgccaggcatcccgggcatcggcggtccgagcggtcctattggcccaccgggtatcccgggcccgaaaggtgaaccgggcctgcctggtccgccaggatttccgggtaagccgggctttccggggccgaagggcgaccgtggtatgggtggtgttccgggtgcgctgggtccgcgtggtgaaaaaggtccgatcggcgctccgggcatcggtggtcctccgggtgaaccgggactcccgggtattccgggtccgatgggtccgccgggtgcgattggttttccgggtccgaaaggtgaaggtggtattgttggtccgcagggtcctccaggtccgaagggcgagccgggtctgcagggttttccggggaaaccgggtttcctgggtgaggttggtccgccgggtatgcgtggtttaccggggccgatcggcccgaagggcgaggcaggtcaaaaaggcgtcccgggtctgcctggcgtgccgggtttgctgggcccgaagggcgagccgggcattccgggcgatcagggcctgcaaggtccgccaggcattccggggatcggtggtccgtccggtcccatcggcccgcctggcatcccgggaccgaagggcgagccgggactgccgggcccgccgggcttcccg

SEQ ID NO: 16 - protein, 141 aa, Homo sapiens
GKPGFPGPKGDRGMGGVPGALGPRGEKGPIGAPGIGGPPGEPGLPGIPGPMGPPGAIGFPGPKGEGGIVGPQGPPGPKGEPGLQGFPGKPGFLGEVGPPGMRGLPGPIGPKGEAGQKGVPGLPGVPGLLGPKGEPGIPGDQ

SEQ ID NO: 17 - protein, 282 aa, synthetic construct
GKPGFPGPKGDRGMGGVPGALGPRGEKGPIGAPGIGGPPGEPGLPGIPGPMGPPGAIGFPGPKGEGGIVGPQGPPGPKGEPGLQGFPGKPGFLGEVGPPGMRGLPGPIGPKGEAGQKGVPGLPGVPGLLGPKGEPGIPGDQGKPGFPGPKGDRGMGGVPGALGPRGEKGPIGAPGIGGPPGEPGLPGIPGPMGPPGAIGFPGPKGEGGIVGPQGPPGPKGEPGLQGFPGKPGFLGEVGPPGMRGLPGPIGPKGEAGQKGVPGLPGVPGLLGPKGEPGIPGDQ

SEQ ID NO: 18 - DNA, 846 bp, synthetic construct
  source 1..846: mol_type = other DNA
gggaaacccggattcccgggtccaaagggtgaccgcggtatgggtggcgtgccgggtgcgctgggtccgcgtggtgagaaaggtccgattggcgctccgggcatcggcggcccaccgggtgaacctggattgccgggcatcccgggtccgatgggtccgccgggagccattggttttccgggtccgaagggtgaaggtggtatcgtgggcccacagggtccgcctgggccgaagggcgaaccgggcctgcagggttttccgggtaaaccgggctttctgggtgaggttggtccgccgggcatgcgtggcctgccgggcccgatcggtccgaagggcgaagcaggtcagaaaggcgtcccgggtctgccgggcgtgccgggcttgctgggcccaaaaggtgagccgggtattccgggggatcagggtaaaccgggcttcccgggtccgaagggtgaccgtggtatgggcggtgtgccgggcgcgctgggtccgcgtggtgaaaaaggccccatcggcgcgccaggcatcggcggcccgccgggcgagccgggcttaccgggtatcccgggcccgatgggtccgccgggtgcgattggtttcccgggcccaaagggcgagggtggtattgttggtccacagggcccaccgggccccaagggtgaaccgggcctgcaaggttttccggggaaaccgggcttcctcggtgaagttggtccgccgggtatgcgcggtctgcctggcccgattggcccaaagggtgaggctggccaaaaaggtgttccgggccttccgggcgtccctggtttgctgggtccgaagggtgagccgggtatcccgggtgatcaa

SEQ ID NO: 19 - protein, 42 aa, Homo sapiens
GKPGFPGPKGDRGMGGVPGALGPRGEKGPIGAPGIGGPPGEP

SEQ ID NO: 20 - protein, 252 aa, synthetic construct
GKPGFPGPKGDRGMGGVPGALGPRGEKGPIGAPGIGGPPGEPGKPGFPGPKGDRGMGGVPGALGPRGEKGPIGAPGIGGPPGEPGKPGFPGPKGDRGMGGVPGALGPRGEKGPIGAPGIGGPPGEPGKPGFPGPKGDRGMGGVPGALGPRGEKGPIGAPGIGGPPGEPGKPGFPGPKGDRGMGGVPGALGPRGEKGPIGAPGIGGPPGEPGKPGFPGPKGDRGMGGVPGALGPRGEKGPIGAPGIGGPPGEP

SEQ ID NO: 21 - DNA, 756 bp, synthetic construct
  source 1..756: mol_type = other DNA
gggaaacccggattcccgggtccgaagggcgatcgcggtatgggcggtgtcccgggagctttgggtccgcgtggtgagaaaggtccgattggtgctccgggtattggtggtccaccgggcgagccgggtaaaccgggcttccctggtccgaagggcgatcgcggcatgggtggcgtgccgggtgcgctgggtccgcgtggtgaaaaaggtccgatcggcgcgccaggcatcggcggaccgcctggcgaacctggcaaaccgggattcccgggcccgaagggtgaccgcggtatgggcggtgttccgggtgcattgggcccgcgtggcgagaagggtccgattggtgcgccagggatcggcggtcctccgggcgagccgggcaaaccgggctttccgggcccgaaaggtgatcgtggcatgggtggtgtgccgggtgcgctgggcccgcgtggtgaaaagggcccgatcggcgccccgggcattggcggtcctccgggcgagccgggcaagccgggttttccgggtcccaagggtgaccgtggtatgggtggtgttccgggtgcgctgggtccgagaggtgagaaagggccgatcggtgcccctggcatcggcggtccgccaggcgaaccggggaaaccgggttttccgggcccaaaaggcgaccgcggtatgggtggtgttccgggtgcgctgggtccgcgtggtgaaaagggcccgatcggcgcaccgggcattggaggcccaccgggcgaaccg

SEQ ID NO: 22 - protein, 42 aa, Homo sapiens
GPKGEGGIVGPQGPPGPKGEPGLQGFPGKPGFLGEVGPPGMR

SEQ ID NO: 23 - protein, 252 aa, synthetic construct
GPKGEGGIVGPQGPPGPKGEPGLQGFPGKPGFLGEVGPPGMRGPKGEGGIVGPQGPPGPKGEPGLQGFPGKPGFLGEVGPPGMRGPKGEGGIVGPQGPPGPKGEPGLQGFPGKPGFLGEVGPPGMRGPKGEGGIVGPQGPPGPKGEPGLQGFPGKPGFLGEVGPPGMRGPKGEGGIVGPQGPPGPKGEPGLQGFPGKPGFLGEVGPPGMRGPKGEGGIVGPQGPPGPKGEPGLQGFPGKPGFLGEVGPPGMR

SEQ ID NO: 24 - DNA, 756 bp, synthetic construct
  source 1..756: mol_type = other DNA
gggcccaaaggagagggcggtatcgtgggcccacagggtccgccgggccccaagggtgaaccgggcctgcaaggctttccgggcaaaccgggtttccttggcgaggttggcccaccgggtatgcgcggtccgaaaggcgagggtggcatcgtgggtccacaaggtccgcctggtccgaagggtgaaccgggcctgcagggtttcccgggtaaacctggctttctgggtgaggttggtccgccgggcatgcgtggtccgaagggcgagggtggtatcgtgggccctcagggtccgccgggtccgaagggcgagccgggtttgcaaggttttccgggcaaaccgggctttctgggtgaggttggtccgccgggcatgcgtggtccgaagggtgagggcggtattgttggtccgcagggcccaccgggcccgaagggtgaaccgggtttacaaggcttcccgggtaaaccgggctttctgggcgaagttggcccaccgggtatgcgtggtccgaaaggcgaaggtggtattgtgggtccgcagggcccaccgggtccgaagggggaaccgggtttgcaaggcttcccgggcaaaccgggattcttgggcgaagtgggcccgccggggatgcgtggtccgaagggtgaaggcggtattgtcggtccgcagggtccgccgggtccaaaaggcgaaccgggcctgcagggcttcccgggtaaaccgggcttcctgggtgaggtcggtccgccgggcatgcgc

SEQ ID NO: 25 - protein, 33 aa, Homo sapiens
GPKGEAGQKGVPGLPGVPGLLGPKGEPGIPGDQ

SEQ ID NO: 26 - protein, 198 aa, synthetic construct
GPKGEAGQKGVPGLPGVPGLLGPKGEPGIPGDQGPKGEAGQKGVPGLPGVPGLLGPKGEPGIPGDQGPKGEAGQKGVPGLPGVPGLLGPKGEPGIPGDQGPKGEAGQKGVPGLPGVPGLLGPKGEPGIPGDQGPKGEAGQKGVPGLPGVPGLLGPKGEPGIPGDQGPKGEAGQKGVPGLPGVPGLLGPKGEPGIPGDQ

SEQ ID NO: 27 - DNA, 594 bp, synthetic construct
  source 1..594: mol_type = other DNA
gggcccaaaggagaggcgggtcagaaaggtgtgccaggcctgccaggcgttccgggtttgctgggtccgaagggtgaaccgggtatcccgggcgatcagggtccgaaaggtgaggcaggtcaaaaaggcgtgccgggcctgccgggtgtgccgggcttgcttggcccgaagggtgaaccgggcatcccgggagatcaaggtcctaaaggcgaagctggccaaaaaggcgtcccaggcctgccgggcgtgccgggtttgctgggtccgaaaggcgagccgggtatcccgggcgaccagggtccgaagggtgaagccggtcagaaaggtgttccgggcctgccgggcgtgccgggtttgctgggcccaaagggcgagccgggcattccgggtgaccagggtccgaagggcgaagcgggtcagaaaggcgttccgggcctgccgggtgttccgggtctgctcggtccgaagggtgagccgggcattccgggcgaccaaggtccgaagggcgaggcgggtcagaaaggtgttccgggtctgcctggcgtcccaggtttactgggtccgaagggtgaaccgggtattccgggcgatcaa

SEQ ID NO: 28 - protein, 39 aa, Homo sapiens
GKPGVAGLHGPPGKPGALGPQGQPGLPGPPGPPGPPGPP

SEQ ID NO: 29 - protein, 234 aa, synthetic construct
GKPGVAGLHGPPGKPGALGPQGQPGLPGPPGPPGPPGPPGKPGVAGLHGPPGKPGALGPQGQPGLPGPPGPPGPPGPPGKPGVAGLHGPPGKPGALGPQGQPGLPGPPGPPGPPGPPGKPGVAGLHGPPGKPGALGPQGQPGLPGPPGPPGPPGPPGKPGVAGLHGPPGKPGALGPQGQPGLPGPPGPPGPPGPPGKPGVAGLHGPPGKPGALGPQGQPGLPGPPGPPGPPGPP

SEQ ID NO: 30 - DNA, 702 bp, synthetic construct
  source 1..702: mol_type = other DNA
gggaaacccggagtcgccggtttgcacggcccaccgggcaaaccgggcgctttgggcccgcagggccaaccgggcctgccaggcccaccgggcccgccgggcccaccgggtccgccgggtaagccgggggtggccggtcttcacggccccccgggtaaaccgggagctctgggtcctcaaggtcaacctggcctgccgggtccgccgggcccgccgggcccaccgggtccgccgggcaagccgggcgtggcaggtctgcacggtccgccggggaaaccgggtgcgctgggtccgcaaggtcaaccgggtttaccgggtccgccgggtccgccgggcccaccgggtccgccgggcaagccgggcgttgcaggtttgcacggcccgccaggcaaaccgggtgcgctgggtccgcagggtcagccgggcctgccgggcccgccgggcccgccaggtccgccgggcccgccgggtaaaccgggtgtggcgggtctgcacggtccgccgggcaagcctggcgcgctgggtccgcagggtcagccgggtctgccgggcccgcctgggccgcccggtccgccgggtccgcctggcaagccgggtgttgcgggtctgcatggtccgccgggcaagccgggtgcgctgggcccgcagggtcagccgggcttgccgggtccgccgggcccgccgggtccaccgggcccgcca